European Patent Application EP 4 269 585 A1, published November 1, 2023. Title: Guide RNA for editing the polyadenylation signal sequence of a target RNA. Applicant: Astellas Pharma Inc. The sequence listing filed with the application follows.

SEQUENCE LISTING (22 sequences)

SEQ ID NO: 1 - DNA, 241 bp, Artificial Sequence
  hU6
gagggcctatttcccatgattccttcatatttgcatatacgatacaaggctgttagagagataattagaattaatttgactgtaaacacaaagatattagtacaaaatacgtgacgtagaaagtaataatttcttgggtagtttgcagttttaaaattatgttttaaaatggactatcatatgcttaccgtaacttgaaagtatttcgatttcttggctttatatatcttgtggaaaggac

SEQ ID NO: 2 - DNA, 95 bp, Artificial Sequence
  U6-ASR-STL
ggtgctcgcttcggcagcacatatactagtcgaccagatgtaatgaaaataaagatattttatcgcgtctagagcggacttcggtccgctttttt

SEQ ID NO: 3 - RNA, 27 nt, Artificial Sequence
  RNA of U6
gugcucgcuucggcagcacauauacua

SEQ ID NO: 4 - DNA, 27 bp, Artificial Sequence
  DNA 0f U6
gtgctcgcttcggcagcacatatacta

SEQ ID NO: 5 - RNA, 20 nt, Artificial Sequence
  RNA of STL
gcggacuucgguccgcuuuu

SEQ ID NO: 6 - DNA, 20 bp, Artificial Sequence
  DNA of STL
gcggacttcggtccgctttt

SEQ ID NO: 7 - DNA, 66 bp, Artificial Sequence
  ASR-Gq
gggcagatgtaatgaaaataaagatattttatcgcggggtttgggtttgggtttgggttttttttt

SEQ ID NO: 8 - DNA, 70 bp, Artificial Sequence
  BoxB-ASR
gggagagggccctgaagagggcccttttctcagatgtaatgaaaataaagatattttatcgcgttttttt

SEQ ID NO: 9 - RNA, 24 nt, Artificial Sequence
  RNA of Gq
ggguuuggguuuggguuuggguuu

SEQ ID NO: 10 - DNA, 24 bp, Artificial Sequence
  DNA of Gq
gggtttgggtttgggtttgggttt

SEQ ID NO: 11 - RNA, 24 nt, Artificial Sequence
  RNA of BoxB
agagggcccugaagagggcccuuu

SEQ ID NO: 12 - DNA, 24 bp, Artificial Sequence
  DNA of BoxB
agagggccctgaagagggcccttt

SEQ ID NO: 13 - DNA, 71 bp, Artificial Sequence
  DNA of Control
gggagagggccctgaagagggcccttttctgaatgcaattgttgttgttaacttgtttatcgcattttttt

SEQ ID NO: 14 - DNA, 591 bp, Artificial Sequence
  Artifical sequence
gcggccgctggccgcaataaaatatctttattttcattacatctgtgctgtgccttctagttgccagccatctgttgtttgcccctcccccgtgccttccttgaccctggaaggtgccactcccactgtcctttcctaataaaatgaggaaattgcatcgcattgtctgagtaggtgtcattctattctggggggtggggtggggcaggacagcaagggggaggattgggaagacaatagcaggcatgctggggatgcggtgggctctatggtgttggttttttgtgtgaggatctaaatgagtcttcggacctcgcgggggccgcttaagcggtggttagggtttgtctgacgcggggggagggggaaggaacgaaacactctcattcggaggcggctcggggtttggtcttggtggccacgggcacgcagaagagcgccgcgatcctcttaagcacccccccgccctccgtggaggcgggggtttggtcggcgggtggtaactggcgggccgctgactcgggcgggtcgcgcgccccagagtgtgaccttttcggtctgctcgcagacccccgggcggcgccgccgcgg

SEQ ID NO: 15 - protein, 701 aa, Artificial Sequence
  Amino Acid of hADAR
MDIEDEENMSSSSTDVKENRNLDNVSPKDGSTPGPGEGSQLSNGGGGGPGRKRPLEEGSNGHSKYRLKKRRKTPGPVLPKNALMQLNEIKPGLQYTLLSQTGPVHAPLFVMSVEVNGQVFEGSGPTKKKAKLHAAEKALRSFVQFPNASEAHLAMGRTLSVNTDFTSDQADFPDTLFNGFETPDKAEPPFYVGSNGDDSFSSSGDLSLSASPVPASLAQPPLPVLPPFPPPSGKNPVMILNELRPGLKYDFLSESGESHAKSFVMSVVVDGQFFEGSGRNKKLAKARAAQSALAAIFNLHLDQTPSRQPIPSEGLQLHLPQVLADAVSRLVLGKFGDLTDNFSSPHARRKVLAGVVMTTGTDVKDAKVISVSTGTKCINGEYMSDRGLALNDCHAEIISRRSLLRFLYTQLELYLNNKDDQKRSIFQKSERGGFRLKENVQFHLYISTSPCGDARIFSPHEPILEEPADRHPNRKARGQLRTKIESGEGTIPVRSNASIQTWDGVLQGERLLTMSCSDKIARWNVVGIQGSLLSIFVEPIYFSSIILGSLYHGDHLSRAMYQRISNIEDLPPLYTLNKPLLSGISNAEARQPGKAPNFSVNWTVGDSAIEVINATTGKDELGRASRLCKHALYCRWMRVHGKVPSHLLRSKITKPNVYHESKLAAKEYQAAKARLFTAFIKAGLGAWVEKPTEQDQFSLTP

SEQ ID NO: 16 - DNA, 2127 bp, Artificial Sequence
  DNA of hADAR2
gaattcgccgccaccatggatatagaagatgaagaaaacatgagttccagcagcactgatgtgaaggaaaaccgcaatctggacaacgtgtcccccaaggatggcagcacacctgggcctggcgagggctctcagctctccaatgggggtggtggtggccccggcagaaagcggcccctggaggagggcagcaatggccactccaagtaccgcctgaagaaaaggaggaaaacaccagggcccgtcctccccaagaacgccctgatgcagctgaatgagatcaagcctggtttgcagtacacactcctgtcccagactgggcccgtgcacgcgcctttgtttgtcatgtctgtggaggtgaatggccaggtttttgagggctctggtcccacaaagaaaaaggcaaaactccatgctgctgagaaggccttgaggtctttcgttcagtttcctaatgcctctgaggcccacctggccatggggaggaccctgtctgtcaacacggacttcacatctgaccaggccgacttccctgacacgctcttcaatggttttgaaactcctgacaaggcggagcctcccttttacgtgggctccaatggggatgactccttcagttccagcggggacctcagcttgtctgcttccccggtgcctgccagcctagcccagcctcctctccctgtcttaccaccattcccacccccgagtgggaagaatcccgtgatgatcttgaacgaactgcgcccaggactcaagtatgactttctctccgagagcggggagagccatgccaagagcttcgtcatgtctgtggtcgtggatggtcagttctttgaaggctcggggagaaacaagaagcttgccaaggcccgggctgcgcagtctgccctggccgccatttttaacttgcacttggatcagacgccatctcgccagcctattcccagtgagggtcttcagctgcatttaccgcaggttttagctgacgctgtctcacgcctggtcctgggtaagtttggtgacctgaccgacaacttctcctcccctcacgctcgcagaaaagtgctggctggagtcgtcatgacaacaggcacagatgttaaagatgccaaggtgataagtgtttctacaggaacaaaatgtattaatggtgaatacatgagtgatcgtggccttgcattaaatgactgccatgcagaaataatatctcggagatccttgctcagatttctttatacacaacttgagctttacttaaataacaaagatgatcaaaaaagatccatctttcagaaatcagagcgaggggggtttaggctgaaggagaatgtccagtttcatctgtacatcagcacctctccctgtggagatgccagaatcttctcaccacatgagccaatcctggaagaaccagcagatagacacccaaatcgtaaagcaagaggacagctacggaccaaaatagagtctggtgaggggacgattccagtgcgctccaatgcgagcatccaaacgtgggacggggtgctgcaaggggagcggctgctcaccatgtcctgcagtgacaagattgcacgctggaacgtggtgggcatccagggatccctgctcagcattttcgtggagcccatttacttctcgagcatcatcctgggcagcctttaccacggggaccacctttccagggccatgtaccagcggatctccaacatagaggacctgccacctctctacaccctcaacaagcctttgctcagtggcatcagcaatgcagaagcacggcagccagggaaggcccccaacttcagtgtcaactggacggtaggcgactccgctattgaggtcatcaacgccacgactgggaaggatgagctgggccgcgcgtcccgcctgtgtaagcacgcgttgtactgtcgctggatgcgtgtgcacggcaaggttccctcccacttactacgctccaagattaccaagcccaacgtgtaccatgagtccaagctggcggcaaaggagtaccaggccgccaaggcgcgtctgttcacagccttcatcaaggcggggctgggggcctgggtggagaagcccaccgagcaggaccagttctcactcacgccctgaagatcc

SEQ ID NO: 17 - DNA, 20 bp, Artificial Sequence
  forward-primer
agcgggaatggctcatatcg

SEQ ID NO: 18 - DNA, 19 bp, Artificial Sequence
  reverse-primer
ggcaccttccagggtcaag

SEQ ID NO: 19 - DNA, 20 bp, Artificial Sequence
  sequence-primer
ggagaagggcgaggttagac

SEQ ID NO: 20 - DNA, 23 bp, Artificial Sequence
  forward-primer(Rluc)
cttcttagctccctcgacaatag

SEQ ID NO: 21 - DNA, 20 bp, Artificial Sequence
  reverse-primer(Rluc)
tccagattgtccgcaactac

SEQ ID NO: 22 - DNA, 25 bp, Artificial Sequence
  probe
ccagcgacgatctgcctaagatgtt